European Patent Application EP 4 806 438 A1, published September 16, 2026. Title: Pharmaceutical combination product comprising an inhibitor of a tyrosine kinase and an autophagy inducer. Applicant: Universität Duisburg-Essen, Körperschaft des öffentlichen Rechts. Application EP. The sequence listing filed with the application follows.

SEQUENCE LISTING (20 sequences)

SEQ ID NO: 1 - protein, 13 aa, Human immunodeficiency virus 1
  VARIANT 1: note = Y or absent
  VARIANT 12: note = P or absent
  VARIANT 13: note = Q or absent
XGRKKRRQRRRXX

SEQ ID NO: 2 - protein, 13 aa, Human immunodeficiency virus 1
  VARIANT 1: note = Q or absent
  VARIANT 2: note = P or absent
  VARIANT 13: note = Y or absent
XXRRRQRRKKRGX

SEQ ID NO: 3 - protein, 450 aa, synthetic construct
MEGSKTSNNSTMQVSFVCQRCSQPLKLDTSFKILDRVTIQELTAPLLTTAQAKPGETQEEETNSGEEPFIETPRQDGVSRRFIPPARMMSTESANSFTLIGEASDGGTMENLSRRLKVTGDLFDIMSGQTDVDHPLCEECTDTLLDQLDTQLNVTENECQNYKRCLEILEQMNEDDSEQLQMELKELALEEERLIQELEDVEKNRKIVAENLEKVQAEAERLDQEEAQYQREYSEFKRQQLELDDELKSVENQMRYAQTQLDKLKKTNVFNATFHIWHSGQFGTINNFRLGRLPSVPVEWNEINAAWGQTVLLLHALANKMGLKFQRYRLVPYGNHSYLESLTDKSKELPLYCSGGLRFFWDNKFDHAMVAFLDCVQQFKEEVEKGETRFCLPYRMDVEKGKIEDTGGSGGSYSIKTQFNSEEQWTKALKFMLTNLKWGLAWVSSQFYNK

SEQ ID NO: 4 - protein, 450 aa, synthetic construct
MEGSKTSNNSTMQVSFVCQRCSQPLKLDTSFKILDRVTIQELTAPLLTTAQAKPGETQEEETNSGEEPFIETPRQDGVSRRFIPPARMMSTESANSFTLIGEASDGGTMENLSRRLKVTGDLFDIMSGQTDVDHPLCEECTDTLLDQLDTQLNVTENECQNYKRCLEILEQMNEDDSEQLQMELKELALEEERLIQELEDVEKNRKIVAENLEKVQAEAERLDQEEAQYQREYSEFKRQQLELDDELKSVENQMRYAQTQLDKLKKTNVFNATFEIWHDGEFGTINNFRLGRLPSVPVEWNEINAAWGQTVLLLHALANKMGLKFQRYRLVPYGNHSYLESLTDKSKELPLYCSGGLRFFWDNKFDHAMVAFLDCVQQFKEEVEKGETRFCLPYRMDVEKGKIEDTGGSGGSYSIKTQFNSEEQWTKALKFMLTNLKWGLAWVSSQFYNK

SEQ ID NO: 5 - protein, 450 aa, synthetic construct
MEGSKTSNNSTMQVSFVCQRCSQPLKLDTSFKILDRVTIQELTAPLLTTAQAKPGETQEEETNSGEEPFIETPRQDGVSRRFIPPARMMSTESANSFTLIGEASDGGTMENLSRRLKVTGDLFDIMSGQTDVDHPLCEECTDTLLDQLDTQLNVTENECQNYKRCLEILEQMNEDDSEQLQMELKELALEEERLIQELEDVEKNRKIVAENLEKVQAEAERLDQEEAQYQREYSEFKRQQLELDDELKSVENQMRYAQTQLDKLKKTNVWNATFHIWHDGQFGTINNFRLGRLPSVPVEWNEINAAWGQTVLLLHALANKMGLKFQRYRLVPYGNHSYLESLTDKSKELPLYCSGGLRFFWDNKFDHAMVAFLDCVQQFKEEVEKGETRFCLPYRMDVEKGKIEDTGGSGGSYSIKTQFNSEEQWTKALKFMLTNLKWGLAWVSSQFYNK

SEQ ID NO: 6 - protein, 450 aa, synthetic construct
MEGSKTSNNSTMQVSFVCQRCSQPLKLDTSFKILDRVTIQELTAPLLTTAQAKPGETQEEETNSGEEPFIETPRQDGVSRRFIPPARMMSTESANSFTLIGEASDGGTMENLSRRLKVTGDLFDIMSGQTDVDHPLCEECTDTLLDQLDTQLNVTENECQNYKRCLEILEQMNEDDSEQLQMELKELALEEERLIQELEDVEKNRKIVAENLEKVQAEAERLDQEEAQYQREYSEFKRQQLELDDELKSVENQMRYAQTQLDKLKKTNVWNATFEIWHDGEFGTINNFRLGRLPSVPVEWNEINAAWGQTVLLLHALANKMGLKFQRYRLVPYGNHSYLESLTDKSKELPLYCSGGLRFFWDNKFDHAMVAFLDCVQQFKEEVEKGETRFCLPYRMDVEKGKIEDTGGSGGSYSIKTQFNSEEQWTKALKFMLTNLKWGLAWVSSQFYNK

SEQ ID NO: 7 - protein, 450 aa, synthetic construct
MEGSKTSNNSTMQVSFVCQRCSQPLKLDTSFKILDRVTIQELTAPLLTTAQAKPGETQEEETNSGEEPFIETPRQDGVSRRFIPPARMMSTESANSFTLIGEASDGGTMENLSRRLKVTGDLFDIMSGQTDVDHPLCEECTDTLLDQLDTQLNVTENECQNYKRCLEILEQMNEDDSEQLQMELKELALEEERLIQELEDVEKNRKIVAENLEKVQAEAERLDQEEAQYQREYSEFKRQQLELDDELKSVENQMRYAQTQLDKLKKTNDHWIHFTANWVGQFGTINNFRLGRLPSVPVEWNEINAAWGQTVLLLHALANKMGLKFQRYRLVPYGNHSYLESLTDKSKELPLYCSGGLRFFWDNKFDHAMVAFLDCVQQFKEEVEKGETRFCLPYRMDVEKGKIEDTGGSGGSYSIKTQFNSEEQWTKALKFMLTNLKWGLAWVSSQFYNK

SEQ ID NO: 8 - protein, 450 aa, synthetic construct
MEGSKTSNNSTMQVSFVCQRCSQPLKLDTSFKILDRVTIQELTAPLLTTAQAKPGETQEEETNSGEEPFIETPRQDGVSRRFIPPARMMSTESANSFTLIGEASDGGTMENLSRRLKVTGDLFDIMSGQTDVDHPLCEECTDTLLDQLDTQLNVTENECQNYKRCLEILEQMNEDDSEQLQMELKELALEEERLIQELEDVEKNRKIVAENLEKVQAEAERLDQEEAQYQREYSEFKRQQLELDDELKSVENQMRYAQTQLDKLKKTNDHWIEFTANWVGEFGTINNFRLGRLPSVPVEWNEINAAWGQTVLLLHALANKMGLKFQRYRLVPYGNHSYLESLTDKSKELPLYCSGGLRFFWDNKFDHAMVAFLDCVQQFKEEVEKGETRFCLPYRMDVEKGKIEDTGGSGGSYSIKTQFNSEEQWTKALKFMLTNLKWGLAWVSSQFYNK

SEQ ID NO: 9 - protein, 18 aa, homo sapiens
TNVFNATFHIWHSGQFGT

SEQ ID NO: 10 - protein, 18 aa, synthetic construct
TNVFNATFEIWHDGEFGT

SEQ ID NO: 11 - protein, 33 aa, synthetic construct
  VARIANT 1: note = Y or absent
  VARIANT 12: note = P or absent
  VARIANT 13: note = Q or absent
  VARIANT 24: note = H or E
  VARIANT 28: note = D or S
  VARIANT 30: note = E or Q
XGRKKRRQRRRXXGGTNVFNATFXIWHXGXFGT

SEQ ID NO: 12 - protein, 33 aa, synthetic construct
  VARIANT 1: note = Q or absent
  VARIANT 2: note = P or absent
  VARIANT 13: note = Y or absent
  VARIANT 24: note = H or E
  VARIANT 28: note = D or S
  VARIANT 30: note = E or Q
XXRRRQRRKKRGXGGTNVFNATFXIWHXGXFGT

SEQ ID NO: 13 - protein, 24 aa, synthetic construct
RRRQRRKKRGYGGDHWIHFTANWV

SEQ ID NO: 14 - protein, 24 aa, synthetic construct
YGRKKRRQRRRGGVWNATFHIWHD

SEQ ID NO: 15 - protein, 10 aa, unidentified
FVNLLFLVVE

SEQ ID NO: 16 - protein, 23 aa, synthetic construct
  VARIANT 1: note = Y or absent
  VARIANT 12: note = P or absent
  VARIANT 13: note = Q or absent
XGRKKRRQRRRXXFVNLLFLVVE

SEQ ID NO: 17 - protein, 23 aa, synthetic construct
  VARIANT 1: note = Q or absent
  VARIANT 2: note = P or absent
  VARIANT 13: note = Y or absent
XXRRRQRRKKRGXFVNLLFLVVE

SEQ ID NO: 18 - protein, 12 aa, unidentified
NEMCYVWHLFTQ

SEQ ID NO: 19 - protein, 25 aa, synthetic construct
  VARIANT 1: note = Y or absent
  VARIANT 12: note = P or absent
  VARIANT 13: note = Q or absent
XGRKKRRQRRRXXNEMCYVWHLFTQ

SEQ ID NO: 20 - protein, 25 aa, synthetic construct
  VARIANT 1: note = Q or absent
  VARIANT 2: note = P or absent
  VARIANT 13: note = Y or absent
XXRRRQRRKKRGXNEMCYVWHLFTQ